European Patent Application EP 4 663 760 A1, published December 17, 2025. Title: MICROORGANISMS FOR PRODUCING L-ALANINE AND PROCESS FOR PRODUCING L-ALANINE USING THE SAME. Applicant: 씨제이제일제당 주식회사. The sequence listing filed with the application follows.

SEQUENCE LISTING (35 sequences)

SEQ ID NO: 1 - protein, 376 aa, Bacillus licheniformis
MIIGIPKEIKNNENRVAITPAGVVALKKSGHQVLIEQGAGLGSGFEDADYKAAGADILAEAKDVWGKADMVMKVKEPISSEYGYFRKGLVLFTYLHLAAEPKLAKALVDSGVTAIAYETVEVNRTLPLLTPMSEVAGRMASQIGAQFLEKSKGGKGILLSGVPGVKRGKVTIIGGGVVGTNAAKIAVGLGADVTLIDLSAERLRQLDDQFGKDIQTLMSNPLNIAEAVKDSDLVIGAVLIPGAKAPKLVTEEMIKSMSPGSVVVDVAIDQGGIIETVDKITTHDDPTYTKHGVVHYAVANMPGAVPRTSTIGLTNVTMPYALQIANKGVEQAVAENQALALGVNVANGSITYKAVARDLGYEYVSVEDAFQTVTAG

SEQ ID NO: 2 - DNA, 1131 bp, Bacillus licheniformis
  source 1..1131: mol_type = genomic DNA
atgatcattggaattcctaaagaaattaaaaacaacgagaaccgtgtagccattactccggccggagtagtcgcgctaaaaaaaagcggtcatcaagttttaattgaacagggagccgggcttggaagcggattcgaggacgccgactacaaagcagccggggcggacattttggctgaagcgaaagatgtgtggggaaaagcggatatggtcatgaaagtgaaagagccgatcagctctgaatacggctatttccgaaaaggacttgttttatttacttatctgcacttagcggctgaacctaagcttgcgaaagcgcttgtggacagcggcgtcacagccatcgcttacgaaacggtcgaagtgaaccggacgcttccgctcttgactccaatgagtgaagtcgccggacgcatggcttcgcagatcggcgcgcaatttcttgagaaatcaaaaggcggcaaaggcatcctgttatcgggcgtacccggtgtaaaacgcggcaaagtcacgatcatcggcggcggagtggttggtacgaacgctgccaaaatcgctgtcggactgggcgctgacgtcactttgatcgacttgagcgctgagcgcctccgtcagctcgatgaccagttcggcaaagacattcaaacgcttatgtccaatccgctcaacattgcggaagccgtaaaagactcagaccttgtcatcggcgccgtcttaattcctggtgcaaaagcgccgaagcttgtcacagaagagatgatcaagtcgatgtcgccaggttcagttgttgtagacgtggcgattgaccagggcggcattatcgaaacggttgataaaatcactacgcatgacgatccgacttacacgaagcacggcgttgtccactatgccgtcgccaatatgccgggagccgttccccgtacatcaacgatcggcttaacaaacgtcaccatgccttacgccttgcaaatcgcaaataaaggcgttgaacaagcagtcgccgaaaatcaggcgctcgctctcggcgtcaacgttgcaaacggaagcatcacctacaaggccgtcgcgcgcgaccttggatatgaatatgtatctgtagaagatgcatttcaaacggtaaccgctggttaa

SEQ ID NO: 3 - protein, 379 aa, Bacillus licheniformis
MIIGVPKEIKNNENRVALTPGAASQLIAAGHRVIVEKDAGTGSGFENEDYVSVGAEISEQAEAVWEAAEMVMKVKEPLPEEYPYFREGLILFTYLHLAAEPSLAEALKQKGVTAIAYETVSNGRSLPLLTPMSEVAGRMAAQIGAQFLEKPKGGKGILLAGVPGVARGKVTIIGGGVVGTNAAKIAAGLGADVTMIDLSADRLRQLDDQFGNQIKTLMSNPVNIADAVAEADLLICAVLIPGAKAPTLVTEEMVKQMKPGSVIVDVAIDQGGIVETVDHITTHDNPTYVKHGVVHYAVANMPGAVPRTSTVALTNVTVPYALEIANKGAEKAILENPALKAGVNTANGHITYEAVARDLNYGYVPAELAIENSSSAAGA

SEQ ID NO: 4 - DNA, 1140 bp, Bacillus licheniformis
  source 1..1140: mol_type = genomic DNA
atgattatcggcgtaccgaaagaaatcaaaaacaatgaaaaccgtgttgctttgactcccggtgcggcttctcaattgatcgcggcaggacaccgcgtcatcgtggaaaaagacgcggggactggaagcgggtttgaaaatgaggattacgtctcagtgggagccgagatctcagaacaggcggaagccgtctgggaagcggctgaaatggtgatgaaagtcaaagagccgctccctgaagaatatccgtattttagagaaggtctcatcttgttcacctacctgcatttagccgcagagccttccttggctgaagcattaaagcagaaaggcgtgacagccatcgcctatgaaaccgtcagcaatggccgttcccttcctttgctgacgccgatgtctgaggtagccgggcggatggccgcccaaatcggcgcgcagttcctcgaaaagccgaaaggcggaaaaggcatattattggccggtgtacccggagtcgcgcgcgggaaagtgacgatcatcggcggaggcgttgtcggcacaaatgcggcaaaaatcgcggcgggcctcggagccgacgtgacgatgatcgatttaagcgcggatcgcctgcgccagcttgatgatcaattcggcaatcaaattaaaacattgatgtccaatccggtcaacatcgccgatgccgtagcggaagccgacctcctcatctgcgcggttctgatcccgggtgccaaagcgccgactttagtgacggaagagatggtcaaacagatgaaaccgggctctgtgattgttgacgtcgcaatcgatcaaggcggcatcgtcgagacggtggatcacatcacaacccacgacaatccgacctatgtcaaacacggagtcgtccattacgctgttgccaacatgcctggcgccgttccgcggacatctacagttgcgctgacgaatgtaacagttccgtatgcgcttgaaatcgcgaacaaaggcgcggaaaaagcgattcttgaaaaccctgcgctaaaagccggcgtcaacacagcaaacggccatattacttatgaagccgtagccagggacttaaactatggctacgttcccgcagagcttgcgatcgaaaattcgtcgtcagccgccggcgcatag

SEQ ID NO: 5 - protein, 376 aa, Bacillus amyloliquefaciens
MIIGVPKEIKNNENRVSLTPGGVSQLIGNGHRVLVESGAGLGSGFTNEDYVSAGAEILEDRKQVWDAEMVMKVKEPLAEEYAYFRQGLILFTYLHLAAEPELAKALTEKGVTAIAYETVTDGRSLPLLTPMSEVAGRMAAQIGAQFLEKPKGGKGILLAGVPGVSRGKVTIIGGGGVGTNAAKMAVGLGADVTMIDLNADRLRQLDDIFGHQIKTLISNPVNIADSVAEADLLICAVLIPGAKAPTLVTEEMVKQMKPGSVIVDVAIDQGGIVETVDHITTHDNPTYEKHGVVHYAVANMPGAVPRTSTLALTNVTVPYALEIANKGAAKAIADSPALKAGLNTANGHVTYEAVAKDLGYDYVPAEKAMRGSAAKA

SEQ ID NO: 6 - DNA, 1131 bp, Bacillus amyloliquefaciens
  source 1..1131: mol_type = genomic DNA
atgattatcggggttccaaaggaaatcaaaaacaatgaaaatcgagtgtcattaacacctggaggcgtttcacagcttatcggaaacggccatcgggttcttgtggaatccggagcaggactcggaagcggctttacaaatgaagattatgtatccgcaggcgcggaaattctggaggacagaaagcaagtttgggatgcagaaatggtcatgaaggtaaaagaaccgctggctgaggagtatgcgtatttccgtcaaggcctgatcttattcacttaccttcatttagccgcagagccggaattagctaaagcgcttacagaaaaaggcgtgacagctattgcgtacgaaacggtaacggacggacgttcacttccgctgcttacgccgatgtctgaagtggccggcagaatggccgctcaaatcggagctcagttccttgaaaaaccaaagggcggaaaaggaattttattagccggcgtaccgggtgtatcccgcggaaaagtcacgatcatcggaggaggcggcgtcggaacaaatgccgcgaaaatggctgtcggactcggtgccgatgtgacgatgatcgacttgaacgcagaccgcctgcgtcagcttgatgatattttcgggcatcagattaaaacattgatctcaaaccctgtaaatattgcagactccgtcgcggaagcggatcttctgatctgtgccgtgctcatcccgggagccaaagcgccgaccctcgttacggaagaaatggttaaacaaatgaaaccgggttccgtcattgttgatgttgccatcgatcagggcggcattgtggaaaccgttgatcatattacaacacacgataatccgacttatgaaaaacacggcgtcgttcattatgctgtcgccaatatgcctggcgccgtaccgcgtacatctacgctcgcattaacgaatgtgaccgttccttacgcgcttgaaatcgccaataaaggcgcggcaaaagccattgcagacagcccggcgcttaaagccggcctgaatacggctaacggacacgtcacgtatgaagcggtagccaaagacttaggctatgactatgtgcctgctgaaaaagcgatgcgaggttcagctgcaaaagcttaa

SEQ ID NO: 7 - protein, 376 aa, Laceyella sacchari
MKVGVPTEIKNNENRVAITPAGVDALVQSGHEVLIQSGAGNGSGFTDDQYATHGAKILGSAKEVWENADMIMKVKEPQPEEVAYFRENLILFTYLHLAPEPELTRALMDKKVAAIAYETIQLDNGALPLLTPMSEVAGRMSVQIGAQFLEKPKGGKGVLLGGVPGVLPGEVVIIGGGVVGTNAAKIALGMGANVTILDINADRLRQLDDQFQGQLRTLMSNRYNLAEAVAKADLLVGAVLIPGRRAPRLVTEEMVRTMQPGSVIVDVAIDQGGSIETIDRVTTHSEPTYVKHGVVHYAVANMPGAVPRTSTIALTNVTIPYAVQIANKGLTQALADNRFLARGVNVINGQVTYSAVAESLGLPYVPLEEAIGQRFA

SEQ ID NO: 8 - DNA, 1131 bp, Laceyella sacchari
  source 1..1131: mol_type = genomic DNA
atgaaagtaggagtgccaacagaaatcaaaaacaatgagaaccgtgtcgccattactccagcgggggtggatgcgctggtgcagtctggccatgaggtgctgatccaaagcggggccggaaatgggagcggtttcacagatgatcagtatgcaacgcatggagccaaaatcttgggcagtgccaaagaagtatgggaaaacgctgacatgatcatgaaagtgaaagaaccgcaaccggaggaggttgcttattttcgggaaaacctaattcttttcacttacctgcatctcgcaccagaaccggagctcacccgggcgttaatggataaaaaagtggctgccatcgcttatgaaacgattcaattggataacggtgcgttgccgttgttgaccccgatgagcgaagtagccggacggatgtcggtgcagatcggggcgcaatttttggagaagcccaaagggggcaaaggggttttgctcggcggcgtccccggggtactgcctggagaagtggtgattatcggtggtggcgtcgtaggtacgaatgcggccaaaatcgctttggggatgggagccaacgtaaccattctcgatattaatgcggatcggttaagacaactggatgaccaattccaaggccagttgcggacgttgatgtccaaccgttacaacttggcggaagccgttgccaaagctgatttgttggtaggcgcggtattgataccaggtcgccgcgcaccgcggttggtgacggaagaaatggttcgcactatgcaacccggttcagtgattgtggatgtggcgatcgaccaaggagggtccattgaaacgatcgaccgggtgacaactcacagtgaaccgacatatgtgaagcacggagtagttcattatgcagtggccaatatgccgggagcggtgccgaggacatcgaccatcgcgttgaccaatgtcacgattccgtacgcagttcagatcgccaacaaaggattgacacaagcacttgccgacaaccgttttctggcacgtggggtgaatgtcatcaatgggcaggtcacctactctgccgtcgccgaaagcttgggtctgccgtatgtgccgctggaagaggcgattggtcaacgctttgcttaa

SEQ ID NO: 9 - DNA, 40 bp, synthetic construct
  source 1..40: mol_type = other DNA
gagatagaggtctttacgtctagaagaaacatcccagcgc

SEQ ID NO: 10 - DNA, 42 bp, synthetic construct
  source 1..42: mol_type = other DNA
ctttaggaattccaatgatcatgagtgtttcctttcgttggg

SEQ ID NO: 11 - DNA, 45 bp, synthetic construct
  source 1..45: mol_type = other DNA
gtacccaacgaaaggaaacactcatgatcattggaattcctaaag

SEQ ID NO: 12 - DNA, 44 bp, synthetic construct
  source 1..44: mol_type = other DNA
gtgaaggaaagagttcctcgagttaaagcagaatggaaaaaagg

SEQ ID NO: 13 - DNA, 40 bp, synthetic construct
  source 1..40: mol_type = other DNA
ctttcggtacgccgataatcatgagtgtttcctttcgttg

SEQ ID NO: 14 - DNA, 41 bp, synthetic construct
  source 1..41: mol_type = other DNA
gtacccaacgaaaggaaacactcatgattatcggcgtaccg

SEQ ID NO: 15 - DNA, 40 bp, synthetic construct
  source 1..40: mol_type = other DNA
gaaggaaagagttcctcgagctgcaattgcggcaaaattg

SEQ ID NO: 16 - DNA, 34 bp, synthetic construct
  source 1..34: mol_type = other DNA
gaaccccgataatcatgagtgtttcctttcgttg

SEQ ID NO: 17 - DNA, 34 bp, synthetic construct
  source 1..34: mol_type = other DNA
caacgaaaggaaacactcatgattatcggggttc

SEQ ID NO: 18 - DNA, 44 bp, synthetic construct
  source 1..44: mol_type = other DNA
gtgaaggaaagagttcctcgagtccgggatatgaattgatattc

SEQ ID NO: 19 - DNA, 45 bp, synthetic construct
  source 1..45: mol_type = other DNA
ctgttggcactcctactttcatgagtgtttcctttcgttgggtac

SEQ ID NO: 20 - DNA, 45 bp, synthetic construct
  source 1..45: mol_type = other DNA
gtacccaacgaaaggaaacactcatgaaagtaggagtgccaacag

SEQ ID NO: 21 - DNA, 38 bp, synthetic construct
  source 1..38: mol_type = other DNA
gaaggaaagagttcctcgaggctccatcgtttcaaacg

SEQ ID NO: 22 - DNA, 36 bp, synthetic construct
  source 1..36: mol_type = other DNA
ctcggtacccggggatccttcccatggaaactctcg

SEQ ID NO: 23 - DNA, 46 bp, synthetic construct
  source 1..46: mol_type = other DNA
gtgtgaaggaaagagttcctcgagtctagacgtaaagacctctatc

SEQ ID NO: 24 - DNA, 46 bp, synthetic construct
  source 1..46: mol_type = other DNA
gagatagaggtctttacgtctagactcgaggaactctttccttcac

SEQ ID NO: 25 - DNA, 34 bp, synthetic construct
  source 1..34: mol_type = other DNA
catgcctgcaggtcgacttgatgagcagcagtgg

SEQ ID NO: 26 - DNA, 29 bp, synthetic construct
  source 1..29: mol_type = other DNA
cacctgggatggcagcaaacttgaacttg

SEQ ID NO: 27 - DNA, 27 bp, synthetic construct
  source 1..27: mol_type = other DNA
caggatgtttgggctggtgaatcatag

SEQ ID NO: 28 - DNA, 45 bp, synthetic construct
  source 1..45: mol_type = other DNA
gagctcggtacccggggatccgttttctacaataaattgagttag

SEQ ID NO: 29 - DNA, 45 bp, synthetic construct
  source 1..45: mol_type = other DNA
caaccggacgcatggcactcgaggcggccgcgaaaaaggctttcg

SEQ ID NO: 30 - DNA, 45 bp, synthetic construct
  source 1..45: mol_type = other DNA
cgaaagcctttttcgcggccgcctcgagtgccatgcgtccggttg

SEQ ID NO: 31 - DNA, 33 bp, synthetic construct
  source 1..33: mol_type = other DNA
catgcctgcaggtcgaccgctcattgggtacgg

SEQ ID NO: 32 - DNA, 40 bp, synthetic construct
  source 1..40: mol_type = other DNA
gaaagcctttttcgcggccgcagaaacatcccagcgctac

SEQ ID NO: 33 - DNA, 42 bp, synthetic construct
  source 1..42: mol_type = other DNA
cttcacaaccggacgcatggcactcgagttaaagcagaatgg

SEQ ID NO: 34 - DNA, 27 bp, synthetic construct
  source 1..27: mol_type = other DNA
cagtcaataggtagtcccgatcccaag

SEQ ID NO: 35 - DNA, 29 bp, synthetic construct
  source 1..29: mol_type = other DNA
gaactaacgaagaaggacgcctaagagac